European Patent Application EP 4 772 644 A1, published July 8, 2026. Title: A microorganism introduced with nicotinamide nucleotide transhydrogenase derived from Edwardsiella tarda and method for producing L-amino acid or derivatives thereof using the same. Applicant: 씨제이제일제당 주식회사. The sequence listing filed with the application follows.

SEQUENCE LISTING (38 sequences)

SEQ ID NO: 1 - DNA, 35 bp, synthetic construct
  source 1..35: mol_type = other DNA
aattcgagctcggtacccaatggagctgaaagaat

SEQ ID NO: 2 - DNA, 30 bp, synthetic construct
  source 1..30: mol_type = other DNA
cttcctgatagtcccgggacattgtttttc

SEQ ID NO: 3 - DNA, 30 bp, synthetic construct
  source 1..30: mol_type = other DNA
gaaaaacaatgtcccgggactatcaggaag

SEQ ID NO: 4 - DNA, 38 bp, synthetic construct
  source 1..38: mol_type = other DNA
gtcgactctagaggatccccataaaaacaggcagagga

SEQ ID NO: 5 - DNA, 35 bp, synthetic construct
  source 1..35: mol_type = other DNA
cctgaaaaacaatgtcccaacgaccgagcctattg

SEQ ID NO: 6 - DNA, 20 bp, synthetic construct
  source 1..20: mol_type = other DNA
gttgtgtctcctctaaagat

SEQ ID NO: 7 - DNA, 34 bp, synthetic construct
  source 1..34: mol_type = other DNA
ctttagaggagacacaacatgcgtattggtgtac

SEQ ID NO: 8 - DNA, 34 bp, synthetic construct
  source 1..34: mol_type = other DNA
ccaacttcctgatagtcccttataatgcgcgtag

SEQ ID NO: 9 - DNA, 32 bp, synthetic construct
  source 1..32: mol_type = other DNA
agaggagacacaacatgcgaattggcatacca

SEQ ID NO: 10 - DNA, 35 bp, synthetic construct
  source 1..35: mol_type = other DNA
aacttcctgatagtcccttacagagctttcaggat

SEQ ID NO: 11 - DNA, 35 bp, synthetic construct
  source 1..35: mol_type = other DNA
tctttagaggagacacaacgtgcgtatcggtattc

SEQ ID NO: 12 - DNA, 38 bp, synthetic construct
  source 1..38: mol_type = other DNA
accaacttcctgatagtcccttagttgctgatccctgc

SEQ ID NO: 13 - DNA, 39 bp, synthetic construct
  source 1..39: mol_type = other DNA
atctttagaggagacacaacatgagaatcggcatccctt

SEQ ID NO: 14 - DNA, 34 bp, synthetic construct
  source 1..34: mol_type = other DNA
ccaacttcctgatagtcccttaagcgttgacctt

SEQ ID NO: 15 - DNA, 37 bp, synthetic construct
  source 1..37: mol_type = other DNA
atctttagaggagacacaacatgcgcatcggtgtgcc

SEQ ID NO: 16 - DNA, 32 bp, synthetic construct
  source 1..32: mol_type = other DNA
acttcctgatagtccctcaacccacccgcagc

SEQ ID NO: 17 - DNA, 472 bp, synthetic construct
  source 1..472: mol_type = other DNA
aacgaccgagcctattgggattaccattgaagccagtgtgagttgcatcacattggcttcaaatctgagactttaatttgtggattcacgggggtgtaatgtagttcataattaaccccattcgggggagcagatcgtagtgcgaacgatttcaggttcgttccctgcaaaaactatttagcgcaagtgttggaaatgcccccgtttggggtcaatgtccatttttgaatgtgtctgtatgattttgcatctgctgcgaaatctttgtttccccgctaaagttgaggacaggttgacacggagttgactcgacgaattatccaatgtgagtaggtttggtgcgtgagttggaaaaattcgccatactcgcccttgggttctgtcagctcaagaattcttgagtgaccgatgctctgattgacctaactgcttgacacattgcatttcctacaatctttagaggagacacaac

SEQ ID NO: 18 - protein, 508 aa, Edwardsiella tarda
MRIGVPKERLANEARVAATPKTVEQLLKLGFTVAIESGAGKLASFEDAAYQQAGAEVVTLDEVWQSDVILKVNAPEDDEIARMKAGTTLISFIWPAQNQPLLDKLAQRQVTVMAMDSVPRISRAQSMDALSSMANIAGYRAIVEAAHEFGRFFTGQITAAGKVPPAKVMVIGAGVAGLAAIGAAGSLGAIVRAFDTRPEVKEQVQSMGAEFLELDFEEEAGSGDGYAKVMSEAFIKAEMALFAAQAQEVDIIVTTALIPGKPAPRLITKEMVATMKSGSVIVDLAAQTGGNCELTQADHVVTTENGVKIIGYTDLPSRLPTQSSQLYATNLVNLLKLLCKEKDGTLHVDFEDVIIRGVTVTQDGEITWPAPAIKVSAQPQAAKVEPVAAVAAKPTSPWRKYLLIALAIVLFGWMASVAPSEFLSHFTVFALSCVVGYYVVWNVSHALHTPLMSVTNAISGIIVVGALLQIGHGGWITFFAFIAVLIASINIFGGFTVTQRMLKMFRKN

SEQ ID NO: 19 - protein, 463 aa, Edwardsiella tarda
MSGGLVTAAYIVAAILFIFSLAGLSKHETSKQGNTFGMVGMAIALIATICGPDAANIGWIIVAMVIGGAIGIYLARKVEMTEMPELVAVLHSFVGLAAVLVGYNSYIEHEPGSMAQVLENIHLVEVFLGVFIGAVTFTGSIVAFGKLRGIISSKPLMLPHRHKLNLAALVVSFLLLLWFVNTGSTGAQVVALLLMTVIALAFGWHLVASIGGADMPVVVSMLNSYSGWAAAAAGFMLSNDLLIVTGALVGSSGAILSYIMCKAMNRSFISVIAGGFGTDGSSTGDEGEMGEYREASAEEVAEMLKNSSSVIITPGYGMAVAQAQYPVAEITQKLRDRGVKVRFGIHPVAGRLPGHMNVLLAEAKVPYDVVLEMDEINDDFADTDTVLVIGANDTVNPAAMEDPRSPIAGMPVLEVWKAQNVIVFKRSMNTGYAGVQNPLFFKENTQMLFGDAKDSVEAILRAL

SEQ ID NO: 20 - protein, 510 aa, Escherichia coli
MRIGIPRERLTNETRVAATPKTVEQLLKLGFTVAVESGAGQLASFDDKAFVQAGAEIVEGNSVWQSEIILKVNAPLDDEIALLNPGTTLVSFIWPAQNPELMQKLAERNVTVMAMDSVPRISRAQSLDALSSMANIAGYRAIVEAAHEFGRFFTGQITAAGKVPPAKVMVIGAGVAGLAAIGAANSLGAIVRAFDTRPEVKEQVQSMGAEFLELDFKEEAGSGDGYAKVMSDAFIKAEMELFAAQAKEVDIIVTTALIPGKPAPKLITREMVDSMKAGSVIVDLAAQNGGNCEYTVPGEIFTTENGVKVIGYTDLPGRLPTQSSQLYGTNLVNLLKLLCKEKDGNITVDFDDVVIRGVTVIRAGEITWPAPPIQVSAQPQAAQKAAPEVKTEEKCTCSPWRKYALMALAIILFGWMASVAPKEFLGHFTVFALACVVGYYVVWNVSHALHTPLMSVTNAISGIIVVGALLQIGQGGWVSFLSFIAVLIASINIFGGFTVTQRMLKMFRKN

SEQ ID NO: 21 - protein, 462 aa, Escherichia coli
MSGGLVTAAYIVAAILFIFSLAGLSKHETSRQGNNFGIAGMAIALIATIFGPDTGNVGWILLAMVIGGAIGIRLAKKVEMTEMPELVAILHSFVGLAAVLVGFNSYLHHDAGMAPILVNIHLTEVFLGIFIGAVTFTGSVVAFGKLCGKISSKPLMLPNRHKMNLAALVVSFLLLIVFVRTDSVGLQVLALLIMTAIALVFGWHLVASIGGADMPVVVSMLNSYSGWAAAAAGFMLSNDLLIVTGALVGSSGAILSYIMCKAMNRSFISVIAGGFGTDGSSTGDDQEVGEHREITAEETAELLKNSHSVIITPGYGMAVAQAQYPVAEITEKLRARGINVRFGIHPVAGRLPGHMNVLLAEAKVPYDIVLEMDEINDDFADTDTVLVIGANDTVNPAAQDDPKSPIAGMPVLEVWKAQNVIVFKRSMNTGYAGVQNPLFFKENTHMLFGDAKASVDAILKAL

SEQ ID NO: 22 - protein, 517 aa, Corynebacterium urealyticum
MRIGIPVEPGENQPLVAATPDTVGKLIKLGYDVEVQAGAGEDAAYPDALYREAGASIVGEEVWEADIVTTLDTPPKEKRDLMRSGATLICRMAPGRNEELINELANRGITGLAMDAVPRISRAQSMDVLSSMANIAGYRAVIEAANAFGRLFTGQVTAAGKVPPAKVYVIGAGVAGLAAIGTANSMGAIVKATDLRVEAGEQVESMGAEFVAIQEEAEKSEDGYAKEMTQDQAELAAKIYSQQSAEADIVITTANIPGRTSPVLLTEEDVANMRPGSVVVDLAAANGGNCALTKPGEVFVTDNGVTIIGYTDLAGRLPGQASQLFGQNIVNLFKLITPEKDGQRVLDLDDEIIRTITVTLNDGQETSVLWPPPPVSVSVAPQQQPAQDTQAAEEPEKQAFMGGPFAKIGLAIAILLGAAIVLVSPLGMSGNFVVLTLAIVLGFYVISAVTPTLHTPLMSETNAISGIVLVGAILQVNSPNIIVTVLAFLAIVVSSVNVFGGFAITDRMLGMFVKEDA

SEQ ID NO: 23 - protein, 495 aa, Corynebacterium urealyticum
MTATLILSQAATGENATLLDWLARISNLAYIVAAVLFLMALAGLSKPETAKRGNTLGMSGMAVAIAVAIFQAVVHSTTDSDALDPVITVVLIALAMSLGAAYGIKRAHSVEMTGLPQLIALFNGMVGLGAVFIGYNSFVSESADSMGAAAYNFHLGEVFLGIFIGAVTFTGSILAGLKLSGKVKGAPLLLPARNLLNVAILVISLVLMVVFILAGEGTTAWIAVGIMTALALFMGWHLVAAIGGGDMPVVVSIMNSYSGWAAAFTGLMLQNPLLIITGALVGSSGAFLSYVMCQAMNRSFLNVLLGGFGTDGGAVAEGVDGTHTEIDTDEAVAMLKDAKNIMITPGYGMAVSQAQYTVAELTRKLRDQGKTVQFGIHPVAGRLPGHMNVLLAEAKVPYDIVMDMEEINDDFDEVDVVLVIGANDTVNPSAEMPGSPIAGMPVLKVWEAERVIVLKRSMGAGYSGAQNPLFFNENTDMLLGDAKASIEKLAAGISN

SEQ ID NO: 24 - protein, 524 aa, Corynebacterium amycolatum
MRIGIPLEPDPQQTIVAATPETVGKLVKLGYDVAVQADAGLAAKFTDADYESAGAAIVDESVWHSDIVVTLDTPPEQFRALLNDGAMLVSRLAPGRNEELVEELAHRNITALAMDAVPRISRAQSMDVLSSMANIGGYRAVVEAASAYGRLFTGQVTAAGKMPPATVYVIGAGVGGLAAIGTANSMGAIVKATDLRPEAGEQVESMGAEFIPIPAATEKSEDGYAKEMTNDQAAAAAKLYSEQSAQADIVITTANIPGRRSPLLLTAADVAAMKPGSVIVDMAAAGGGNCEMTVPGKTIVTDNGVTIIGYTDLAGRLPAQASSLYGQNIFNLFKLITPEKDGSPVLNLEDEIIRGITVTKARPQNGAGATGAEILWPPPPIKVAVTPAAPLQEQQAQQAALEENAPEKVSFMGSGMGSKIALGLTALLAIVVMLSAPHSVSANFMVLTLAIVLGFYVISAVTPRLHTPLMSETNAISGIVLVGAILQVGSSNLLVSGLAFAAIVVSSINIFGGFAVTDRMLGMF

SEQ ID NO: 25 - protein, 491 aa, Corynebacterium amycolatum
MASIDTASLLDWTYRLSNVGYIVAAVLFLAALSGLSKPETARRGNAFGIAGMAVAVVIAIFQALVTADTKPDSHFSPLITLILIAVAIGIGGVIGISRARSVAMTGMPQLIALFNGLVGLGAIFIGFNSYIFAEDVAPDALKFHFGEVYIGVFIGAVTFTGSIVAGLKLSEKIKGSPLLLPGRNALNIAILVVTLVLLAVFIATGTEGGAIAWACMVAVTALGLFLGWHLVIAIGGGDMPVVVSIMNSYSGWAAAFTGLMLGNPLLIITGALVGSSGAYLSYIMCEAMNRSFANVILGGFGSEASSGSAVEGSHTEVSHEDTSEILRDADKILIAPGYGMAVAQAQYAVADLVRNLRDAGKEVVFGIHPVAGRLPGHMNVLLAEAKVPYDIVLELDEVNDDFADVDVTLVIGANDTVNPMAEQPGSPIAGMPVLKVWESERVIVLKRSMGSGYSGVQNPLFFNENTDMLIGDAKASIDSLNRILADSKVNA

SEQ ID NO: 26 - protein, 535 aa, Cellulosimicrobium funkei
MRIGVPREVRDGERLVAATPRTVERLRALGYDVVVEHDAGAGATFSDAAYEAAGAAVVDAAAAWGADVVTAVNAPTDAQVALLRPGATLVAMLGPANDPDLVQRLAAHGVTALALDAVPRISRAQALDVLSTLSNVAGYRAVVEAAGEYGGMFAGQVTAAGKTPPARVFVIGGGVAGLAAVGAAASLGAQVRAFDVRSEAAEQIESMGGTAVREPAAQQGMSADGYAKPLTPEQEAAALAVYAREAAEADVVITTALVRGRAPRTLTAEAVAGMRPGSVVVDLAASGGGNCALTVPGERVVTEDGVVVVGWTDLAGRLPQHTSQLLGTNVVHLLELLTPGKDGTLALDLDDPVQRGMTVARDGDVLWPPPPVAVSAAPAPGSTVPPPPPDPAQEAADRERAAAEAASAASLRRRRRTVGAALAAVLVTLALSFAPPSLVGHVTVFTLAVVVGYYVISNVTHSLHTPLMAQTNAISGIILVGALLQIGSDDWVVTTLALLAATVASINIFGGFLVANRMIRMFRKDAPARAQGVAR

SEQ ID NO: 27 - protein, 470 aa, Cellulosimicrobium funkei
MTATSVAQAVYVLAAVLFVLSLAGLSKQESARRGNLLGMVGMVLALAATIVLALGTSARPVLVTALLIALVLLVGAAVGTWRARRVEMTQMPELIAILHSFVGAAAVLVGFNSYLTAHAAGADDVAHLVEVSLGVLVGAVTFTGSVVAFLKLSGRTRSAPLQLPGRNLLNLAALLVSLGLVVWFVVAPSIWPLLLLTVVSLALGWHLVASIGGGDMPVVVSMLNSYSGWAAAAAGFMLGNDLLIVTGALVGSSGAILSYIMCKAMNRSFVSVILGGFGAEEGAAPAGGGEGPQGEHREVSADEVAALLRDARSVVITPGYGMAVAKAQYPVAELVELLRDGGAEVRFGVHPVAGRLPGHMNVLLAEARVPYDIVLEMDEINDDLAGTDVVLVIGANDTVNPAALDDPGSPIAGMPVLHVWEAGQVVVFKRSMAAGYAGVQNPLFFRENTGMLFGDAKQRVEDIVAALRVG

SEQ ID NO: 28 - DNA, 1527 bp, Edwardsiella tarda
  source 1..1527: mol_type = other DNA
atgcgtattggtgtaccaaaagagcggttggccaatgaagcccgcgtagcagcgacgccgaagacggtcgaacaactgcttaaactgggtttcacggtggctatcgagagcggggccggcaagctggccagttttgaggatgcagcctatcaacaggctggcgccgaagtggttacgttggatgaggtgtggcagagtgatgtgatcctcaaggtcaatgcgccggaggatgacgagattgcgcgcatgaaggccggtacgacgttgatcagctttatctggccggcgcagaatcagccgttgctcgataagctcgcacagcgtcaggtgacggtgatggcgatggattcggtgccgcgtatttcacgcgctcagtcgatggatgccctgagctcaatggccaatatcgccggttaccgagctatcgtggaggcggcgcatgagtttggccgtttctttaccgggcagatcacggcagcgggtaaagtcccgccggcgaaagtgatggtgattggggccggtgtcgccgggttggccgccatcggtgccgccgggagcctgggggcgattgtgcgcgccttcgatactcgtccagaagtgaaggagcaggtgcagagtatgggcgccgagttcctcgaactggatttcgaagaggaggcgggcagtggcgatggctatgccaaggtgatgtctgaggctttcatcaaggcggagatggcactgttcgccgcccaggcacaagaggtcgatatcatcgtcaccacggcgttgattccgggcaagccagcaccgcgtttgatcaccaaagagatggtcgccaccatgaaatcggggagtgtcatcgtcgatctggcggcacagaccggtggtaactgcgagctgacgcaggccgaccacgtcgtgaccacggagaatggcgttaagattatcggttataccgatttgcctagccgcttgcctacacagtcttcccagctgtatgccaccaacctggttaacttgctcaagctattgtgtaaagagaaggatgggacgctacacgtggacttcgaggatgtcatcatccgcggggtaaccgtgacgcaggacggggagattacctggccggcaccagcgattaaggtctccgcacaaccacaggcggcgaaagtcgaacctgtcgctgccgtggccgccaaaccgacctcaccgtggcggaagtatctgctgatcgccttggccattgtgttgtttggctggatggccagcgtggcgccgagtgagtttctctcccactttaccgtcttcgcgctctcctgcgtggtggggtactacgtggtgtggaatgtgagccatgcgttgcatacaccgctgatgtcggtcacgaatgcaatctctggcatcatcgtggtcggtgcgctgttgcagattgggcatggcggttggatcaccttctttgcctttattgcggtgttgatcgccagtatcaacatcttcggtggtttcaccgtcacccagcgcatgttgaaaatgtttcgcaagaactga

SEQ ID NO: 29 - DNA, 1392 bp, Edwardsiella tarda
  source 1..1392: mol_type = other DNA
atgtctggaggattagtaaccgcagcatacattgttgccgccatcctgtttatttttagtctggctggcttgtccaagcatgagacatcgaagcagggtaacaccttcggtatggtcggtatggccatcgccctgatcgcgaccatctgtggccctgacgccgcaaacatcggttggatcatcgtggcgatggtgatcgggggggctatcggtatctatctggcgcgcaaggttgaaatgaccgagatgccggagctggttgccgtgctgcatagcttcgtcggtttggccgccgtcctggtaggttacaatagctatatcgagcatgagccgggcagtatggcgcaggtgctggagaacatccatctggtggaggttttcctcggcgtcttcatcggtgccgtgacctttaccgggtcgatcgtcgcgtttggtaaactacgcggtatcatttcgtccaagccgttgatgctgcctcatcgccacaagctgaatctggcggcgttggtcgtctcattcctgttgctattgtggtttgtgaacaccggatctaccggcgcgcaggtcgttgccttgttgctgatgaccgtgatcgcactggccttcggctggcacttggtggcctccatcggcggtgccgacatgccggtcgtggtgtcgatgttgaactcctattcgggttgggccgcggcggccgccggctttatgctgagcaacgatctgctgatcgtcaccggcgcgttggtcggttcttccggtgccatcctctcttacatcatgtgtaaggcgatgaatcgctccttcatcagcgtaatcgccggtggtttcgggaccgatggttcgtcgacgggcgatgaaggtgagatgggcgaataccgtgaggcgagcgccgaagaggtggccgagatgctgaagaactcctcgtcggtcatcatcaccccgggctatggtatggccgtcgctcaggctcagtatccggtagccgagatcacccagaagctgcgcgatcgtggtgtgaaggtgcgtttcggtatccacccggtcgcggggcgactgcctggccatatgaacgtgctactggccgaggccaaggtgccttatgacgtggtgctggagatggacgagatcaacgatgatttcgccgatacggatacggtgctggttatcggtgctaacgacacggtcaacccggcggcgatggaggatccccgtagtccgatcgcggggatgccggtattggaggtgtggaaggcgcaaaacgtcatcgtgttcaagcgctcaatgaataccggttatgccggggttcagaacccgctgttctttaaagagaatactcagatgctgttcggcgatgccaaggatagcgtcgaggcgattctacgcgcattataa

SEQ ID NO: 30 - DNA, 1533 bp, Escherichia coli
  source 1..1533: mol_type = other DNA
atgcgaattggcataccaagagaacggttaaccaatgaaacccgtgttgcagcaacgccaaaaacagtggaacagctgctgaaactgggttttaccgtcgcggtagagagcggcgcgggtcaactggcaagttttgacgataaagcgtttgtgcaagcgggcgctgaaattgtagaagggaatagcgtctggcagtcagagatcattctgaaggtcaatgcgccgttagatgatgaaattgcgttactgaatcctgggacaacgctggtgagttttatctggcctgcgcagaatccggaattaatgcaaaaacttgcggaacgtaacgtgaccgtgatggcgatggactctgtgccgcgtatctcacgcgcacaatcgctggacgcactaagctcgatggcgaacatcgccggttatcgcgccattgttgaagcggcacatgaatttgggcgcttctttaccgggcaaattactgcggccgggaaagtgccaccggcaaaagtgatggtgattggtgcgggtgttgcaggtctggccgccattggcgcagcaaacagtctcggcgcgattgtgcgtgcattcgacacccgcccggaagtgaaagaacaagttcaaagtatgggcgcggaattcctcgagctggattttaaagaggaagctggcagcggcgatggctatgccaaagtgatgtcggacgcgttcatcaaagcggaaatggaactctttgccgcccaggcaaaagaggtcgatatcattgtcaccaccgcgcttattccaggcaaaccagcgccgaagctaattacccgtgaaatggttgactccatgaaggcgggcagtgtgattgtcgacctggcagcccaaaacggcggcaactgtgaatacaccgtgccgggtgaaatcttcactacggaaaatggtgtcaaagtgattggttataccgatcttccgggccgtctgccgacgcaatcctcacagctttacggcacaaacctcgttaatctgctgaaactgttgtgcaaagagaaagacggcaatatcactgttgattttgatgatgtggtgattcgcggcgtgaccgtgatccgtgcgggcgaaattacctggccggcaccgccgattcaggtatcagctcagccgcaggcggcacaaaaagcggcaccggaagtgaaaactgaggaaaaatgtacctgctcaccgtggcgtaaatacgcgttgatggcgctggcaatcattctttttggctggatggcaagcgttgcgccgaaagaattccttgggcacttcaccgttttcgcgctggcctgcgttgtcggttattacgtggtgtggaatgtatcgcacgcgctgcatacaccgttgatgtcggtcaccaacgcgatttcagggattattgttgtcggagcactgttgcagattggccagggcggctgggttagcttccttagttttatcgcggtgcttatagccagcattaatattttcggtggcttcaccgtgactcagcgcatgctgaaaatgttccgcaaaaattaa

SEQ ID NO: 31 - DNA, 1389 bp, Escherichia coli
  source 1..1389: mol_type = other DNA
atgtctggaggattagttacagctgcatacattgttgccgcgatcctgtttatcttcagtctggccggtctttcgaaacatgaaacgtctcgccagggtaacaacttcggtatcgccgggatggcgattgcgttaatcgcaaccatttttggaccggatacgggtaatgttggctggatcttgctggcgatggtcattggtggggcaattggtatccgtctggcgaagaaagttgaaatgaccgaaatgccagaactggtggcgatcctgcatagcttcgtgggtctggcggcagtgctggttggctttaacagctatctgcatcatgacgcgggaatggcaccgattctggtcaatattcacctgacggaagtgttcctcggtatcttcatcggggcggtaacgttcacgggttcggtggtggcgttcggcaaactgtgtggcaagatttcgtctaaaccattgatgctgccaaaccgtcacaaaatgaacctggcggctctggtcgtttccttcctgctgctgattgtatttgttcgcacggacagcgtcggcctgcaagtgctggcattgctgataatgaccgcaattgcgctggtattcggctggcatttagtcgcctccatcggtggtgcagatatgccagtggtggtgtcgatgctgaactcgtactccggctgggcggctgcggctgcgggctttatgctcagcaacgacctgctgattgtgaccggtgcgctggtcggttcttcgggggctatcctttcttacattatgtgtaaggcgatgaaccgttcctttatcagcgttattgcgggtggtttcggcaccgacggctcttctactggcgatgatcaggaagtgggtgagcaccgcgaaatcaccgcagaagagacagcggaactgctgaaaaactcccattcagtgatcattactccggggtacggcatggcagtcgcgcaggcgcaatatcctgtcgctgaaattactgagaaattgcgcgctcgtggtattaatgtgcgtttcggtatccacccggtcgcggggcgtttgcctggacatatgaacgtattgctggctgaagcaaaagtaccgtatgacatcgtgctggaaatggacgagatcaatgatgactttgctgataccgataccgtactggtgattggtgctaacgatacggttaacccggcggcgcaggatgatccgaagagtccgattgctggtatgcctgtgctggaagtgtggaaagcgcagaacgtgattgtctttaaacgttcgatgaacactggctatgctggtgtgcaaaacccgctgttcttcaaggaaaacacccacatgctgtttggtgacgccaaagccagcgtggatgcaatcctgaaagctctgtaa

SEQ ID NO: 32 - DNA, 1554 bp, Corynebacterium urealyticum
  source 1..1554: mol_type = other DNA
gtgcgtatcggtattccggttgagccgggtgagaaccagccgctggtggcagccacaccagacacggtcggcaagctcatcaagcttggctatgacgttgaagtacaggcaggtgccggcgaagacgccgcctaccctgacgccctctaccgcgaggccggcgcgagcatcgtaggcgaggaggtctgggaagcggacatcgtcacgacgctcgacaccccgcccaaggagaagcgcgacctcatgcgctccggagccaccctgatctgccgcatggctccaggccgcaacgaggagctcatcaacgagctcgccaaccgtggcatcaccgggctcgcgatggacgctgtgccgcgtatttcccgcgcacagtccatggatgtcctctcctccatggcaaacatcgccggctaccgcgcagtcatcgaggccgccaacgccttcggtcgactgttcaccggccaggtcaccgcggcaggtaaggtgccgccggcaaaggtctacgtcatcggcgctggtgtcgctggcctggccgcgatcggtaccgccaactccatgggcgcgatcgtcaaggccaccgacctgcgcgtcgaggcaggcgagcaggtcgagtccatgggggcggaattcgtcgccatccaggaagaggccgagaagtccgaggacggctacgccaaggagatgacccaagaccaggcggaactcgctgcgaagatctattcccagcagtccgccgaagccgacatcgtcatcaccaccgcaaacattccgggccgcacctcgccggtgctgctcaccgaggaagatgtcgccaacatgcgtccgggcagcgtcgtcgtcgacctggcggcagccaacggtggtaactgcgcgctgacgaagccgggcgaggtcttcgtcaccgataacggcgtgaccatcattggctacaccgacctggcgggccgcctgcctggccaggcctcccagctgttcggccagaacatcgtcaacctgttcaagctgatcacgccggagaaggacggccagcgcgtgctggacctggatgacgagatcatccgcaccatcaccgtcaccctcaatgacggccaggagacctccgtcctctggccgccaccaccggtgagcgtgtccgtcgccccgcagcagcagcccgcgcaggacacgcaggccgccgaggagccggagaagcaagccttcatgggtggccccttcgccaagatcggtctggccatcgccatcctactgggcgctgcaatcgtcctggtcagcccgctgggaatgagcggcaacttcgtcgtcctgaccctggccatcgtgctgggcttctacgtgatctccgctgtcaccccgaccctgcacaccccgttgatgtccgagacgaacgcgatttcaggaatcgtcctggtcggcgcgatcttgcaggtcaacagccccaatatcatcgttacggtcctcgcgttcctggcaatcgtcgtgtcctccgtcaacgtgttcggtggcttcgccatcacagaccgcatgctcggcatgttcgttaaggaggatgcataa

SEQ ID NO: 33 - DNA, 1488 bp, Corynebacterium urealyticum
  source 1..1488: mol_type = other DNA
atgactgccactctgattctttcgcaggcagcgaccggcgagaacgccacgctgctggattggctggcccggatctcgaacctggcctacatcgtggctgccgtgctcttcctcatggcactggccggcctctctaagccggagaccgcaaagcgcggtaacacgctgggcatgagcggtatggctgttgccatcgccgtggccatcttccaggccgtggttcactccaccaccgattccgatgccctggacccggtcatcaccgtcgtcctcattgccctggctatgagcctcggtgcggcctacggcatcaagcgcgcgcactccgtcgagatgactggtctgccgcagctgatcgcgctgttcaacggcatggtcggtctgggcgcggtcttcatcggctacaactccttcgtttccgagtccgccgactcgatgggtgctgccgcctacaacttccacctgggtgaggtcttcctcggcatcttcatcggtgccgtgaccttcaccggctcgatcctggctggcctgaagctctccggcaaggtcaagggcgccccgctgctgctgccggcccgtaacctgctgaacgtcgccatcctggtgatcagcctcgtgctcatggtcgtgttcatcctcgcgggtgaaggcaccaccgcctggatcgcggttggcatcatgaccgccctggcgctgttcatgggctggcacctggtcgctgccattggcggtggcgacatgccggtcgtcgtgtccatcatgaactcctactccggctgggcagctgccttcaccggtctgatgctgcagaacccgctgctgatcatcaccggtgcgctggtcggttcctccggtgcattcctctcctacgtgatgtgccaggcgatgaaccgctccttcctgaacgtcctgctgggcggcttcggcaccgacggtggcgcggtcgcggagggtgtcgacggcacccacaccgagatcgacaccgacgaggctgtcgcgatgctcaaggacgcgaagaacatcatgatcaccccgggctacggcatggctgtctcccaagcgcagtacacggtcgctgagctgacccgcaagctgcgcgaccagggtaagactgtccagttcggtatccacccggtcgccggtcgcctgcctggccacatgaacgtcctgctggctgaggcgaaggtcccttatgacatcgtcatggatatggaggagatcaacgacgacttcgacgaggtcgacgtggtcctggtcatcggcgcgaacgatacggtcaacccgagcgctgagatgccgggctccccgatcgccggcatgccggttctgaaggtgtgggaggctgagcgcgtgatcgtgctgaagcgttccatgggtgccggttactccggtgcgcagaacccgctgttcttcaacgagaacaccgacatgctgctcggtgatgcgaaggcatccatcgagaagctggccgcagggatcagcaactaa

SEQ ID NO: 34 - DNA, 1590 bp, Corynebacterium amycolatum
  source 1..1590: mol_type = other DNA
atgagaatcggcatccctttagaacccgatccccagcaaacaattgtggctgcgaccccggagaccgtcggcaaactcgtcaagcttggctacgacgtcgccgtgcaggctgacgccggcctggctgcaaagttcaccgacgcggactacgaatccgcaggtgccgccattgtcgacgagtctgtctggcacagcgatatcgtcgtaacgctcgacactccgccggagcagttccgcgcactgcttaacgacggcgccatgctggtcagccgacttgcgccaggccgtaacgaagagctggtcgaagagctcgcgcaccgcaacatcactgcccttgctatggacgcagttccccgcatctcccgggcacagtcgatggacgtgctgtcgtcgatggccaacatcggcggctaccgcgcagtagtcgaagcggcttctgcatatggtcgccttttcactggtcaggtgactgccgcaggcaagatgccgccagctaccgtttacgtcatcggcgctggtgtcggcggacttgccgcaatcggtaccgccaactctatgggcgcgattgtcaaggcaacagacctgcgccctgaagccggtgaacaggtcgaatcgatgggtgcagagttcatcccgattccggccgccactgagaagtccgaagatggctacgccaaggaaatgaccaatgatcaggctgccgctgccgcgaagctctactccgagcagtccgcgcaagctgacattgtcatcaccaccgcgaatatcccgggccgtcgctctccgctgctgctgactgctgccgatgttgcagctatgaaaccaggcagcgtcatcgtcgacatggctgccgccggtggcggtaactgcgagatgacagttccaggcaagaccattgtcactgacaacggtgtgaccatcatcggttacaccgaccttgcagggcgtctgcctgcgcaggcatcgtcgctgtacggtcagaacattttcaacctgttcaagctgattacgccagaaaaggatggctctccagttctcaatctcgaggacgagattatccgtggcatcacggtgacaaaggctcgcccacagaatggcgccggcgctaccggagctgagattctctggccaccaccgcccatcaaggtcgctgtcacccctgctgccccgctgcaggaacagcaggctcagcaggctgcattagaagagaatgctccggagaaggtttccttcatgggatcgggcatgggctcgaagattgctctgggcctgacggcactgctggcaattgtggttatgctcagcgcaccgcacagcgtgagcgccaacttcatggttctcaccttggctatcgtgcttggcttctacgtgatctctgcggtcacgccgcgcctgcacacaccgctgatgtctgagaccaacgcgatttccggcattgttctggtgggtgcgattctccaggtgggaagctccaacctgttagtttccggtctcgcgttcgcggccatcgtagtcagctccatcaatatcttcggcggtttcgccgtcaccgaccgcatgcttggcatgttcgtgaaagaggaggcataa

SEQ ID NO: 35 - DNA, 1476 bp, Corynebacterium amycolatum
  source 1..1476: mol_type = other DNA
atggctagcattgatactgcttcgcttctggactggacctaccgcctgtccaacgtcggctacattgtcgccgccgtcctgttcctcgctgcactctcgggcctgtccaagccggagaccgctcgccgcggaaacgccttcggtattgccggcatggccgtcgccgttgtcatcgccatcttccaggcactcgttaccgctgacaccaagccggattctcacttctccccgctgattaccctgattctcatcgctgtcgctatcggcatcggtggtgtcatcggtatcagtcgcgcacgcagcgttgccatgactggtatgccgcagctgattgcactgttcaacggtctggttggactcggcgctatcttcatcggcttcaactcctacatcttcgccgaagatgtcgcccccgatgccctgaagttccacttcggcgaggtttacattggcgtcttcatcggcgccgtgactttcactggctccatcgtcgcaggcctgaagctgtctgagaagatcaagggctcgccgctactgctgccgggccgcaacgctctgaacattgccattctggtggtcactctggttctcctggctgtcttcatcgcaaccggcaccgagggcggcgccatcgcatgggcatgcatggttgcagtcactgctttgggcctgttcttgggctggcacctggtcatcgccatcggtggcggcgatatgccggttgtcgtgtccatcatgaactcgtactccgggtgggccgctgctttcaccggtctcatgcttggcaacccgctgctcatcatcactggtgcgctggttggttcctccggcgcctacctgtcgtacatcatgtgtgaggccatgaaccgctcctttgccaacgttattctgggtggctttggctccgaggcttcgtcgggaagcgccgtggaaggctcccacaccgaggtcagccacgaggacacctccgagattctgcgtgacgcagacaagattctcatcgctccgggctacggtatggctgtggcacaggctcagtacgctgttgctgacctggtccgtaatctgcgtgacgccggcaaggaagtggtcttcggtatccacccagtcgctggccgcctgccgggtcacatgaacgtgctgttggcagaggccaaggttccctacgacatcgtgctggagctggacgaggtcaacgatgatttcgctgatgtggatgtcaccctggtcatcggcgcaaatgacaccgtcaacccgatggcagagcagccgggctccccgattgcgggtatgccggtgctgaaggtgtgggaatctgagcgcgtgattgttctcaagcggtcgatgggttcgggctactcgggcgtgcagaacccgctgttcttcaacgaaaacaccgacatgcttatcggcgatgcgaaggccagcatcgactccctgaatcgcatcctggcggattcgaaggtcaacgcttaa

SEQ ID NO: 36 - DNA, 1608 bp, Cellulosimicrobium funkei
  source 1..1608: mol_type = other DNA
atgcgcatcggtgtgccccgtgaagtacgggatggtgaacggctcgtagccgctactccgcgtaccgtagaacgtcttcgcgccctgggctatgacgtcgtggtcgagcacgatgccggagcgggcgccacgttctcggatgctgcttacgaggctgcaggtgcggcggtggtggatgctgccgcggcttggggcgctgatgtcgttactgccgtgaatgcccccactgacgcacaggttgccttgctgcggcctggtgccacgctggtcgccatgctcggccctgcgaatgaccccgaccttgtacaacggcttgccgcccatggtgttaccgcattggctttggacgcggtcccacgtatttctcgcgcacaagccttggacgtcctgagcacgctctctaacgttgcgggctaccgggcggtggtcgaggcagccggcgagtacggtggaatgtttgctggacaggttactgcagcgggaaaaaccccgcccgcccgggttttcgtgattggaggcggtgttgcgggccttgcagcagttggcgctgcggcatctttgggcgcccaagtgcgcgcgttcgacgtacggtcggaggccgcggaacagatcgagtctatgggcggtacggcagtgcgtgagcctgcggcccagcagggaatgtcggcagacggctatgcgaaaccgttgaccccagagcaggaagcagccgctctggcggtgtatgctcgtgaggcagccgaagcagatgtcgtcatcacgaccgcgctcgtacgcggccgtgctccccggacgctgaccgcagaagcagtggctggcatgcgtcccggtagcgtagtggtagacttggctgcttcaggaggaggtaactgtgcgctcaccgttcccggagagcgggttgtaactgaggacggcgtggtggtagtcggctggaccgacttggcaggtcgtcttcctcagcacacctcacaacttctgggaacgaacgtagtgcatcttctcgaactcctcaccccaggtaaggacggaaccttggccctggatttggacgatcctgtgcaacgtggtatgactgtggcgcgcgatggagatgtgttgtggcctccgccccctgtcgctgtatcggcagctcctgcacccggcagcacggtgcctccgccgccacccgaccctgcccaagaagctgcagatcgcgaacgcgcagccgccgaagccgcatccgctgcctctctgcgtcgtcgccgtcgtaccgttggcgctgcactcgccgcagtccttgtcacgcttgccttgtccttcgcgccgccgtcgttggtcggccatgtcactgttttcacgctggccgttgtagtaggttactatgtaatttccaatgttacccattccttgcacacccccctcatggcccagactaacgctatttcaggaattattttggttggtgcgctgcttcaaattggatccgacgactgggtcgtcactactcttgccctgctcgctgccactgtagcctctattaacattttcggcggattcttggtggctaaccgcatgatccggatgttccggaaagacgctccagcgcgcgcacagggagttgctcggtga

SEQ ID NO: 37 - DNA, 1413 bp, Cellulosimicrobium funkei
  source 1..1413: mol_type = other DNA
atgaccgcgacctcggtagcccaggcggtctacgtccttgccgctgtcttgttcgtcctgtcactggccggactgtcaaagcaggaaagcgcacggcgcggtaaccttttgggtatggtcggaatggttcttgcacttgctgcgaccattgtactggctctcggcacgtctgcacggccagttctcgtgactgcattgctgatcgccttggttcttctggtaggtgcggctgtaggtacttggcgcgcgcgtcgtgtggaaatgactcagatgcccgagttgattgccattctgcatagctttgtgggtgctgcagctgtgcttgtgggcttcaacagctacttgaccgctcatgcggcaggtgcagatgatgttgcgcacctggtggaggtcagcctcggcgtactggtaggtgctgtgacctttacgggttctgtagtcgcatttcttaagttgtccggtcgcactcggtctgcgccactccaactcccaggtcggaatctccttaatctcgcggcattgctggttagcttgggacttgttgtatggtttgttgttgctccctccatttggccgcttctgttgctgactgttgtaagcttggcgctcggctggcaccttgtggctagcattggaggtggcgacatgccggtagtcgtgtctatgctcaacagctattccggctgggcggcagcggcagcaggatttatgctgggtaacgacctgcttattgttactggagcccttgtcggttcttccggagcaattcttagctatatcatgtgtaaggctatgaatcggtctttcgtgtcggttattctgggcggcttcggtgctgaggagggtgctgcccctgcgggaggcggagagggaccacagggcgaacaccgggaagtttcagccgacgaagttgctgcgttgttgcgggatgcccgctcggttgtcattaccccgggctacggcatggctgtggcaaaagcacagtatccggtcgcagaacttgtggaattgttgcgcgacggcggagctgaggtccggttcggagttcaccctgtggcaggccggctgccaggccacatgaatgtcctgctggcggaagcacgcgtcccatatgatattgttctcgaaatggacgagatcaatgacgaccttgctggcaccgacgtggtgctggttattggtgcgaatgacaccgtgaacccggcggctcttgatgatccgggttcgccgattgccggtatgccggtgcttcacgtatgggaagcaggccaggtagtcgttttcaaacgttccatggctgccggatacgcaggcgtccagaaccctttgttcttccgtgaaaatacgggaatgcttttcggtgacgctaaacaacgggtagaggacatcgtcgctgcgctgcgggtgggttga

SEQ ID NO: 38 - DNA, 5802 bp, synthetic construct
  source 1..5802: mol_type = other DNA
gttcgcttgctgtccataaaaccgcccagtctagctatcgccatgtaagcccactgcaagctacctgctttctctttgcgcttgcgttttcccttgtccagatagcccagtagctgacattcatccggggtcagcaccgtttctgcggactggctttctacgtgttccgcttcctttagcagcccttgcgccctgagtgcttgcggcagcgtgaagctagcttttatcgccattcgccattcaggctgcgcaactgttgggaagggcgatcggtgcgggcctcttcgctattacgccagctggcgaaagggggatgtgctgcaaggcgattaagttgggtaacgccagggttttcccagtcacgacgttgtaaaacgacggccagtgaattcgagctcggtacccggggatcctctagagtcgacctgcaggcatgcaagcttggcgtaatcatggtcatagctgtttcctgtgtgaaattgttatccgctcacaattccacacaacatacgagccggaagcataaagtgtaaagcctggggtgcctaatgagtgagctaactcacattaattgcgttgcgctcactgcccgctttccagtcgggaaacctgtcgtgccagctgcattaatgaatcggccaacgcgcggggagaggcggtttgcgtattgggcgctcttccgcttcctcgctcactgactcgctgcgctcggtcgttcggctgcggcgagcggtatcagctcactcaaaggcggtaatacggttatccacagaatcaggggataacgcaggaaagaacatgtgagcaaaaggccagcaaaaggccaggaaccgtaaaaaggccgcgttgctggcgtttttccataggctccgcccccctgacgagcatcacaaaaatcgacgctcaagtcagaggtggcgaaacccgacaggactataaagataccaggcgtttccccctggaagctccctcgtgcgctctcctgttccgaccctgccgcttaccggatacctgtccgcctttctcccttcgggaagcgtggcgctttctcaatgctcacgctgtaggtatctcagttcggtgtaggtcgttcgctccaagctgggctgtgtgcacgaaccccccgttcagcccgaccgctgcgccttatccggtaactatcgtcttgagtccaacccggtaagacacgacttatcgccactggcagcagccactggtaacaggattagcagagcgaggtatgtaggcggtgctacagagttcttgaagtggtggcctaactacggctacactagaaggacagtatttggtatctgcgctctgctgaagccagttaccttcggaaaaagagttggtagctcttgatccggcaaacaaaccaccgctggtagcggtggtttttttgtttgcaagcagcagattacgcgcagaaaaaaaggatctcaagaagatcctttgatcttttctacggggtctgacgctcagtggaacgaaaactcacgttaagggattttggtcatgagattatcaaaaaggatcttcacctagatccttttggggtgggcgaagaactccagcatgagatccccgcgctggaggatcatccagccctgatagaaacagaagccactggagcacctcaaaaacaccatcatacactaaatcagtaagttggcagcatcacccgacgcactttgcgccgaataaatacctgtgacggaagatcacttcgcagaataaataaatcctggtgtccctgttgataccgggaagccctgggccaacttttggcgaaaatgagacgttgatcggcacgtaagaggttccaactttcaccataatgaaataagatcactaccgggcgtattttttgagttatcgagattttcaggagctgatagaaacagaagccactggagcacctcaaaaacaccatcatacactaaatcagtaagttggcagcatcacccgacgcactttgcgccgaataaatacctgtgacggaagatcacttcgcagaataaataaatcctggtgtccctgttgataccgggaagccctgggccaacttttggcgaaaatgagacgttgatcggcacgtaagaggttccaactttcaccataatgaaataagatcactaccgggcgtattttttgagttatcgagattttcaggagctctttggcatcgtctctcgcctgtcccctcagttcagtaatttcctgcatttgcctgtttccagtcggtagatattccacaaaacagcagggaagcagcgcttttccgctgcataaccctgcttcggggtcattatagcgattttttcggtatatccatcctttttcgcacgatatacaggattttgccaaagggttcgtgtagactttccttggtgtatccaacggcgtcagccgggcaggataggtgaagtaggcccacccgcgagcgggtgttccttcttcactgtcccttattcgcacctggcggtgctcaacgggaatcctgctctgcgaggctggccggctaccgccggcgtaacagatgagggcaagcggatggctgatgaaaccaagccaaccaggaagggcagcccacctatcaaggtgtactgccttccagacgaacgaagagcgattgaggaaaaggcggcggcggccggcatgagcctgtcggcctacctgctggccgtcggccagggctacaaaatcacgggcgtcgtggactatgagcacgtccgcgagggcgtcccggaaaacgattccgaagcccaacctttcatagaaggcggcggtggaatcgaaatctcgtgatggcaggttgggcgtcgcttggtcggtcatttcgaaaaaggttaggaatacggttagccatttgcctgcttttatatagttcatatgggattcacctttatgttgataagaaataaaagaaaatgccaataggatatcggcattttcttttgcgtttttatttgttaactgttaattgtccttgttcaaggatgctgtctttgacaacagatgttttcttgcctttgatgttcagcaggaagctcggcgcaaacgttgattgtttgtctgcgtagaatcctctgtttgtcatatagcttgtaatcacgacattgtttcctttcgcttgaggtacagcgaagtgtgagtaagtaaaggttacatcgttaggcggatcaagatccatttttaacacaaggccagttttgttcagcggcttgtatgggccagttaaagaattagaaacataaccaagcatgtaaatatcgttagacgtaatgccgtcaatcgtcatttttgatccgcgggagtcagtgaacaggtaccatttgccgttcattttaaagacgttcgcgcgttcaatttcatctgttactgtgttagatgcaatcagcggtttcatcacttttttcagtgtgtaatcatcgtttagctcaatcataccgagagcgccgtttgctaactcagccgtgcgttttttatcgctttgcagaagtttttgactttcttgacggaagaatgatgtgcttttgccatagtatgctttgttaaataaagattcttcgccttggtagccatcttcagttccagtgtttgcttcaaatactaagtatttgtggcctttatcttctacgtagtgaggatctctcagcgtatggttgtcgcctgagctgtagttgccttcatcgatgaactgctgtacattttgatacgtttttccgtcaccgtcaaagattgatttataatcctctacaccgttgatgttcaaagagctgtctgatgctgatacgttaacttgtgcagttgtcagtgtttgtttgccgtaatgtttaccggagaaatcagtgtagaataaacggatttttccgtcagatgtaaatgtggctgaacctgaccattcttgtgtttggtcttttaggatagaatcatttgcatcgaatttgtcgctgtctttaaagacgcggccagcgtttttccagctgtcaatagaagtttcgccgactttttgatagaacatgtaaatcgatgtgtcatccgcatttttaggatctccggctaatgcaaagacgatgtggtagccgtgatagtttgcgacagtgccgtcagcgttttgtaatggccagctgtcccaaacgtccaggccttttgcagaagagatatttttaattgtggacgaatcaaattcagaaacttgatatttttcatttttttgctgttcagggatttgcagcatatcatggcgtgtaatatgggaaatgccgtatgtttccttatatggcttttggttcgtttctttcgcaaacgcttgagttgcgcctcctgccagcagtgcggtagtaaaggttaatactgttgcttgttttgcaaactttttgatgttcatcgttcatgtctccttttttatgtactgtgttagcggtctgcttcttccagccctcctgtttgaagatggcaagttagttacgcacaataaaaaaagacctaaaatatgtaaggggtgacgccaaagtatacactttgccctttacacattttaggtcttgcctgctttatcagtaacaaacccgcgcgatttacttttcgacctcattctattagactctcgtttggattgcaactggtctattttcctcttttgtttgatagaaaatcataaaaggatttgcagactacgggcctaaagaactaaaaaatctatctgtttcttttcattctctgtattttttatagtttctgttgcatgggcataaagttgcctttttaatcacaattcagaaaatatcataatatctcatttcactaaataatagtgaacggcaggtatatgtgatgggttaaaaaggatcaccccagagtcccgctcagaagaactcgtcaagaaggcgatagaaggcgatgcgctgcgaatcgggagcggcgataccgtaaagcacgaggaagcggtcagcccattcgccgccaagctcttcagcaatatcacgggtagccaacgctatgtcctgatagcggtccgccacacccagccggccacagtcgatgaatccagaaaagcggccattttccaccatgatattcggcaagcaggcatcgccatgggtcacgacgagatcctcgccgtcgggcatccgcgccttgagcctggcgaacagttcggctggcgcgagcccctgatgctcttcgtccagatcatcctgatcgacaagaccggcttccatccgagtacgtgctcgctcgatgcgatgtttcgcttggtggtcgaatgggcaggtagccggatcaagcgtatgcagccgccgcattgcatcagccatgatggatactttctcggcaggagcaaggtgagatgacaggagatcctgccccggcacttcgcccaatagcagccagtcccttcccgcttcagtgacaacgtcgagacagctgcgcaaggaacgcccgtcgtggccagccacgatagccgcgctgcctcgtcttggagttcattcagggcaccggacaggtcggtcttgacaaaaagaaccgggcgcccctgcgctgacagccggaacacggcggcatcagagcagccgattgtctgttgtgcccagtcatagccgaatagcctctccacccaagcggccggagaacctgcgtgcaatccatcttgttcaatcatgcgaaacgatcctcatcctgtctcttgatcagatcttgatcccctgcgccatcagatccttggcggcaagaaagccatccagtttactttgcagggcttcccaaccttaccagagggcgccccagctggcaattccg